European Patent Application EP 4 775 268 A2, published July 15, 2026. Title: ANTI-CORONAVIRUS POLYPEPTIDE AS WELL AS DERIVATIVE AND APPLICATION THEREOF. Applicant: Institute of Microbiology, Chinese Academy of Sciences. Application US. The sequence listing filed with the application follows.

SEQUENCE LISTING (17 sequences)

SEQ ID NO: 1 - protein, 35 aa, synthetic construct
ISGINASVVNIQKEIDRLNEVAKNLNESLIDLKEL

SEQ ID NO: 2 - protein, 40 aa, synthetic construct
VDLGDISGINASVVNIQKEIDRLNEVAKNLNESLIDLQEL

SEQ ID NO: 3 - protein, 40 aa, synthetic construct
VKFGDISGINASVVNIKEEIDRLYEVVKNLNESLIDLQEL

SEQ ID NO: 4 - protein, 35 aa, synthetic construct
ISGINASVVNIQKEIDRLNEVAKNLNESLIDLQEL

SEQ ID NO: 5 - protein, 41 aa, synthetic construct
ISGINASVVNIQKEIDRLNEVAKNLNESLIDLKELGSGSGC

SEQ ID NO: 6 - protein, 46 aa, synthetic construct
VDLGDISGINASVVNIQKEIDRLNEVAKNLNESLIDLQELGSGSGC

SEQ ID NO: 7 - protein, 46 aa, synthetic construct
VKFGDISGINASVVNIKEEIDRLYEVVKNLNESLIDLQELGSGSGC

SEQ ID NO: 8 - protein, 35 aa, synthetic construct
SVVNIKEEIDRLYEVVKNLNESLIDLQELGSGSGC

SEQ ID NO: 9 - protein, 36 aa, synthetic construct
ISGINASVVNIQKEIDRLNEVAKNLNESLIDLKELC

SEQ ID NO: 10 - protein, 41 aa, synthetic construct
VDLGDISGINASVVNIQKEIDRLNEVAKNLNESLIDLQELC

SEQ ID NO: 11 - protein, 41 aa, synthetic construct
VKFGDISGINASVVNIKEEIDRLYEVVKNLNESLIDLQELC

SEQ ID NO: 12 - protein, 39 aa, synthetic construct
DLGDISGINASVVNIQKEIDRLNEVAKNLNESLIDLQEL

SEQ ID NO: 13 - protein, 38 aa, synthetic construct
LGDISGINASVVNIQKEIDRLNEVAKNLNESLIDLQEL

SEQ ID NO: 14 - protein, 37 aa, synthetic construct
GDISGINASVVNIQKEIDRLNEVAKNLNESLIDLQEL

SEQ ID NO: 15 - protein, 45 aa, synthetic construct
DLGDISGINASVVNIQKEIDRLNEVAKNLNESLIDLQELGSGSGC

SEQ ID NO: 16 - protein, 44 aa, synthetic construct
LGDISGINASVVNIQKEIDRLNEVAKNLNESLIDLQELGSGSGC

SEQ ID NO: 17 - protein, 43 aa, synthetic construct
GDISGINASVVNIQKEIDRLNEVAKNLNESLIDLQELGSGSGC